European Patent Application EP 4 299 738 A1, published January 3, 2024. Title: Semi-rational approach to genome evolutionary engineering in plants. Applicant: Kobe University. The sequence listing filed with the application follows.

SEQUENCE LISTING (29 sequences)

SEQ ID NO: 1 - DNA, 1997 bp, Zea mays
ctgcagtgcagcgtgacccggtcgtgcccctctctagagataatgagcattgcatgtctaagttataaaaaattaccacatattttttttgtcacacttgtttgaagtgcagtttatctatctttatacatatatttaaactttactctacgaataatataatctatagtactacaataatatcagtgttttagagaatcatataaatgaacagttagacatggtctaaaggacaattgagtattttgacaacaggactctacagttttatctttttagtgtgcatgtgttctcctttttttttgcaaatagcttcacctatataatacttcatccattttattagtacatccatttagggtttagggttaatggtttttatagactaatttttttagtacatctattttattctattttagcctctaaattaagaaaactaaaactctattttagtttttttatttaataatttagatataaaatagaataaaataaagtgactaaaaattaaacaaataccctttaagaaattaaaaaaactaaggaaacatttttcttgtttcgagtagataatgccagcctgttaaacgccgtcgacgagtctaacggacaccaaccagcgaaccagcagcgtcgcgtcgggccaagcgaagcagacggcacggcatctctgtcgctgcctctggacccctctggagagttccgctccaccgttggacttgctccgctgtcggcatccagaaattgcgtggcggagcggcagacgtgagccggcacggcaggcggcctcctcctcctctcacggcaccggcagctacgggggattcctttcccaccgctccttcgctttcccttcctcgcccgccgtaataaatagacaccccctccacaccctctttccccaacctcgtgttgttcggagcgcacacacacacaaccagatctcccccaaatccacccgtcggcacctccgcttcaaggtacgccgctcgtcctccccccccccccctctctaccttctctagatcggcgttccggtccatggttagggcccggtagttctacttctgttcatgtttgtgttagatccgtgtttgtgttagatccgtgctgctagcgttcgtacacggatgcgacctgtacgtcagacacgttctgattgctaacttgccagtgtttctctttggggaatcctgggatggctctagccgttccgcagacgggatcgatttcatgattttttttgtttcgttgcatagggtttggtttgcccttttcctttatttcaatatatgccgtgcacttgtttgtcgggtcatcttttcatgcttttttttgtcttggttgtgatgatgtggtctggttgggcggtcgttctagatcggagtagaattaattctgtttcaaactacctggtggatttattaattttggatctgtatgtgtgtgccatacatattcatagttacgaattgaagatgatggatggaaatatcgatctaggataggtatacatgttgatgcgggttttactgatgcatatacagagatgctttttgttcgcttggttgtgatgatgtggtgtggttgggcggtcgttcattcgttctagatcggagtagaatactgtttcaaactacctggtgtatttattaattttggaactgtatgtgtgtgtcatacatcttcatagttacgagtttaagatggatggaaatatcgatctaggataggtatacatgttgatgtgggttttactgatgcatatacatgatggcatatgcagcatctattcatatgctctaaccttgagtacctatctattataataaacaagtatgttttataattattttgatcttgatatacttggatgatggcatatgcagcagctatatgtggatttttttagccctgccttcatacgctatttatttgcttggtactgtttcttttgtcgatgctcaccctgttgtttggtgttacttctgcag

SEQ ID NO: 2 - DNA, 4116 bp, Artificial Sequence
  dCas9
atggataagaagtactctatcggactcgctatcggaactaactctgtgggatgggctgtgatcaccgatgagtacaaggtgccatctaagaagttcaaggttctcggaaacaccgataggcactctatcaagaaaaaccttatcggtgctctcctcttcgattctggtgaaactgctgaggctaccagactcaagagaaccgctagaagaaggtacaccagaagaaagaacaggatctgctacctccaagagatcttctctaacgagatggctaaagtggatgattcattcttccacaggctcgaagagtcattcctcgtggaagaagataagaagcacgagaggcaccctatcttcggaaacatcgttgatgaggtggcataccacgagaagtaccctactatctaccacctcagaaagaagctcgttgattctactgataaggctgatctcaggctcatctacctcgctctcgctcacatgatcaagttcagaggacacttcctcatcgagggtgatctcaaccctgataactctgatgtggataagttgttcatccagctcgtgcagacctacaaccagcttttcgaagagaaccctatcaacgcttcaggtgtggatgctaaggctatcctctctgctaggctctctaagtcaagaaggcttgagaacctcattgctcagctccctggtgagaagaagaacggacttttcggaaacttgatcgctctctctctcggactcacccctaacttcaagtctaacttcgatctcgctgaggatgcaaagctccagctctcaaaggatacctacgatgatgatctcgataacctcctcgctcagatcggagatcagtacgctgatttgttcctcgctgctaagaacctctctgatgctatcctcctcagtgatatcctcagagtgaacaccgagatcaccaaggctccactctcagcttctatgatcaagagatacgatgagcaccaccaggatctcacacttctcaaggctcttgttagacagcagctcccagagaagtacaaagagattttcttcgatcagtctaagaacggatacgctggttacatcgatggtggtgcatctcaagaagagttctacaagttcatcaagcctatcctcgagaagatggatggaaccgaggaactcctcgtgaagctcaatagagaggatcttctcagaaagcagaggaccttcgataacggatctatccctcatcagatccacctcggagagttgcacgctatccttagaaggcaagaggatttctacccattcctcaaggataacagggaaaagattgagaagattctcaccttcagaatcccttactacgtgggacctctcgctagaggaaactcaagattcgcttggatgaccagaaagtctgaggaaaccatcaccccttggaacttcgaagaggtggtggataagggtgctagtgctcagtctttcatcgagaggatgaccaacttcgataagaaccttccaaacgagaaggtgctccctaagcactctttgctctacgagtacttcaccgtgtacaacgagttgaccaaggttaagtacgtgaccgagggaatgaggaagcctgcttttttgtcaggtgagcaaaagaaggctatcgttgatctcttgttcaagaccaacagaaaggtgaccgtgaagcagctcaaagaggattacttcaagaaaatcgagtgcttcgattcagttgagatttctggtgttgaggataggttcaacgcatctctcggaacctaccacgatctcctcaagatcattaaggataaggatttcttggataacgaggaaaacgaggatatcttggaggatatcgttcttaccctcaccctctttgaagatagagagatgattgaagaaaggctcaagacctacgctcatctcttcgatgataaggtgatgaagcagttgaagagaagaagatacactggttggggaaggctctcaagaaagctcattaacggaatcagggataagcagtctggaaagacaatccttgatttcctcaagtctgatggattcgctaacagaaacttcatgcagctcatccacgatgattctctcacctttaaagaggatatccagaaggctcaggtttcaggacagggtgatagtctccatgagcatatcgctaacctcgctggatctcctgcaatcaagaagggaatcctccagactgtgaaggttgtggatgagttggtgaaggtgatgggaaggcataagcctgagaacatcgtgatcgaaatggctagagagaaccagaccactcagaagggacagaagaactctagggaaaggatgaagaggatcgaggaaggtatcaaagagcttggatctcagatcctcaaagagcaccctgttgagaacactcagctccagaatgagaagctctacctctactacctccagaacggaagggatatgtatgtggatcaagagttggatatcaacaggctctctgattacgatgttgatgctatcgtgccacagtcattcttgaaggatgattctatcgataacaaggtgctcaccaggtctgataagaacaggggtaagagtgataacgtgccaagtgaagaggttgtgaagaaaatgaagaactattggaggcagctcctcaacgctaagctcatcactcagagaaagttcgataacttgactaaggctgagaggggaggactctctgaattggataaggcaggattcatcaagaggcagcttgtggaaaccaggcagatcactaagcacgttgcacagatcctcgattctaggatgaacaccaagtacgatgagaacgataagttgatcagggaagtgaaggttatcaccctcaagtcaaagctcgtgtctgatttcagaaaggatttccaattctacaaggtgagggaaatcaacaactaccaccacgctcacgatgcttaccttaacgctgttgttggaaccgctctcatcaagaagtatcctaagctcgagtcagagttcgtgtacggtgattacaaggtgtacgatgtgaggaagatgatcgctaagtctgagcaagagatcggaaaggctaccgctaagtatttcttctactctaacatcatgaatttcttcaagaccgagattaccctcgctaacggtgagatcagaaagaggccactcatcgagacaaacggtgaaacaggtgagatcgtgtgggataagggaagggatttcgctaccgttagaaaggtgctctctatgccacaggtgaacatcgttaagaaaaccgaggtgcagaccggtggattctctaaagagtctatcctccctaagaggaactctgataagctcattgctaggaagaaggattgggaccctaagaaatacggtggtttcgattctcctaccgtggcttactctgttctcgttgtggctaaggttgagaagggaaagagtaagaagctcaagtctgttaaggaacttctcggaatcactatcatggaaaggtcatctttcgagaagaacccaatcgatttcctcgaggctaagggatacaaagaggttaagaaggatctcatcatcaagctcccaaagtactcactcttcgaactcgagaacggtagaaagaggatgctcgcttctgctggtgagcttcaaaagggaaacgagcttgctctcccatctaagtacgttaactttctttacctcgcttctcactacgagaagttgaagggatctccagaagataacgagcagaagcaacttttcgttgagcagcacaagcactacttggatgagatcatcgagcagatctctgagttctctaaaagggtgatcctcgctgatgcaaacctcgataaggtgttgtctgcttacaacaagcacagagataagcctatcagggaacaggcagagaacatcatccatctcttcacccttaccaacctcggtgctcctgctgctttcaagtacttcgatacaaccatcgataggaagagatacacctctaccaaagaagtgctcgatgctaccctcatccatcagtctatcactggactctacgagactaggatcgatctctcacagctcggtggtgattcaagggctgat

SEQ ID NO: 3 - DNA, 51 bp, Artificial Sequence
  dCas9 N-terminal nuclear transport signal
atggctcctaagaagaagcggaaggttggtattcacggggtgcctgcggct

SEQ ID NO: 4 - DNA, 21 bp, Artificial Sequence
  dCas9 C-terminal nuclear transport signal
cctaagaagaagaggaaggtt

SEQ ID NO: 5 - DNA, 4116 bp, Artificial Sequence; identical to SEQ ID NO: 2
  nCas9

SEQ ID NO: 6 - DNA, 1017 bp, Artificial Sequence
  modified UNG1 gene
caaactacgatcgaagacttctttggtacaaagaaaagcactaatgaggcgcccaataagaaaggtaaatcgggcgctactttcatgaccataacaaatggcgcagctatcaagacagagacaaaggcggtcgcaaaggaggcaaacacggacaaatatcctgctaattcaaatgcaaaagatgtatattcgaagaacttgagcagcaatttacgtacactactgtcgctggagctagaaacgattgatgattcgtggtttccacatttaatggatgaatttaaaaagccatattttgtaaagttgaaacagtttgtcactaaagagcaagctgatcatacagtatttccgcctgcaaaggatatttactcatggaccaggctaacgccttttaataaagttaaagtcgtgattatcggtcaagatccctaccacaactttaatcaggcgcatggcttggcttttagcgtcaaaccccctacaccagcaccaccgtcattaaagaacatatataaggaactgaagcaagagtatcctgattttgttgaagataataaagtgggagatttaactcactgggcttcacaaggggttttattgcttgatacctcgttaactgtaagagcacataatgcaaactcgcattctaagcatggttgggaaacttttacaaaaagggtagttcagttgttgatccaggacagagaggccgacggtaagagtttagtattcctcttatgggggaacaatgctatcaaattagtagagtctctgttgggatctacttccgttggaagcggtagtaagtaccctaatatcatggtgatgaagtcagtgcatccgtctccattaagtgcaagttgtggattttttggtaccaaccatttcaaaatgataaacgattggctatacaatacccgcggagagaaaatgatagactggagtgttgttcctggaacgtcattaagagaagttcaggaggcaaatgctcgcttagagtcagaatcaaaggaccct

SEQ ID NO: 7 - DNA, 5409 bp, Artificial Sequence
  dCas9-UNG1 expression unit (d1)
atggctcctaagaagaagcggaaggttggtattcacggggtgcctgcggctatggataagaagtactctatcggactcgctatcggaactaactctgtgggatgggctgtgatcaccgatgagtacaaggtgccatctaagaagttcaaggttctcggaaacaccgataggcactctatcaagaaaaaccttatcggtgctctcctcttcgattctggtgaaactgctgaggctaccagactcaagagaaccgctagaagaaggtacaccagaagaaagaacaggatctgctacctccaagagatcttctctaacgagatggctaaagtggatgattcattcttccacaggctcgaagagtcattcctcgtggaagaagataagaagcacgagaggcaccctatcttcggaaacatcgttgatgaggtggcataccacgagaagtaccctactatctaccacctcagaaagaagctcgttgattctactgataaggctgatctcaggctcatctacctcgctctcgctcacatgatcaagttcagaggacacttcctcatcgagggtgatctcaaccctgataactctgatgtggataagttgttcatccagctcgtgcagacctacaaccagcttttcgaagagaaccctatcaacgcttcaggtgtggatgctaaggctatcctctctgctaggctctctaagtcaagaaggcttgagaacctcattgctcagctccctggtgagaagaagaacggacttttcggaaacttgatcgctctctctctcggactcacccctaacttcaagtctaacttcgatctcgctgaggatgcaaagctccagctctcaaaggatacctacgatgatgatctcgataacctcctcgctcagatcggagatcagtacgctgatttgttcctcgctgctaagaacctctctgatgctatcctcctcagtgatatcctcagagtgaacaccgagatcaccaaggctccactctcagcttctatgatcaagagatacgatgagcaccaccaggatctcacacttctcaaggctcttgttagacagcagctcccagagaagtacaaagagattttcttcgatcagtctaagaacggatacgctggttacatcgatggtggtgcatctcaagaagagttctacaagttcatcaagcctatcctcgagaagatggatggaaccgaggaactcctcgtgaagctcaatagagaggatcttctcagaaagcagaggaccttcgataacggatctatccctcatcagatccacctcggagagttgcacgctatccttagaaggcaagaggatttctacccattcctcaaggataacagggaaaagattgagaagattctcaccttcagaatcccttactacgtgggacctctcgctagaggaaactcaagattcgcttggatgaccagaaagtctgaggaaaccatcaccccttggaacttcgaagaggtggtggataagggtgctagtgctcagtctttcatcgagaggatgaccaacttcgataagaaccttccaaacgagaaggtgctccctaagcactctttgctctacgagtacttcaccgtgtacaacgagttgaccaaggttaagtacgtgaccgagggaatgaggaagcctgcttttttgtcaggtgagcaaaagaaggctatcgttgatctcttgttcaagaccaacagaaaggtgaccgtgaagcagctcaaagaggattacttcaagaaaatcgagtgcttcgattcagttgagatttctggtgttgaggataggttcaacgcatctctcggaacctaccacgatctcctcaagatcattaaggataaggatttcttggataacgaggaaaacgaggatatcttggaggatatcgttcttaccctcaccctctttgaagatagagagatgattgaagaaaggctcaagacctacgctcatctcttcgatgataaggtgatgaagcagttgaagagaagaagatacactggttggggaaggctctcaagaaagctcattaacggaatcagggataagcagtctggaaagacaatccttgatttcctcaagtctgatggattcgctaacagaaacttcatgcagctcatccacgatgattctctcacctttaaagaggatatccagaaggctcaggtttcaggacagggtgatagtctccatgagcatatcgctaacctcgctggatctcctgcaatcaagaagggaatcctccagactgtgaaggttgtggatgagttggtgaaggtgatgggaaggcataagcctgagaacatcgtgatcgaaatggctagagagaaccagaccactcagaagggacagaagaactctagggaaaggatgaagaggatcgaggaaggtatcaaagagcttggatctcagatcctcaaagagcaccctgttgagaacactcagctccagaatgagaagctctacctctactacctccagaacggaagggatatgtatgtggatcaagagttggatatcaacaggctctctgattacgatgttgatgctatcgtgccacagtcattcttgaaggatgattctatcgataacaaggtgctcaccaggtctgataagaacaggggtaagagtgataacgtgccaagtgaagaggttgtgaagaaaatgaagaactattggaggcagctcctcaacgctaagctcatcactcagagaaagttcgataacttgactaaggctgagaggggaggactctctgaattggataaggcaggattcatcaagaggcagcttgtggaaaccaggcagatcactaagcacgttgcacagatcctcgattctaggatgaacaccaagtacgatgagaacgataagttgatcagggaagtgaaggttatcaccctcaagtcaaagctcgtgtctgatttcagaaaggatttccaattctacaaggtgagggaaatcaacaactaccaccacgctcacgatgcttaccttaacgctgttgttggaaccgctctcatcaagaagtatcctaagctcgagtcagagttcgtgtacggtgattacaaggtgtacgatgtgaggaagatgatcgctaagtctgagcaagagatcggaaaggctaccgctaagtatttcttctactctaacatcatgaatttcttcaagaccgagattaccctcgctaacggtgagatcagaaagaggccactcatcgagacaaacggtgaaacaggtgagatcgtgtgggataagggaagggatttcgctaccgttagaaaggtgctctctatgccacaggtgaacatcgttaagaaaaccgaggtgcagaccggtggattctctaaagagtctatcctccctaagaggaactctgataagctcattgctaggaagaaggattgggaccctaagaaatacggtggtttcgattctcctaccgtggcttactctgttctcgttgtggctaaggttgagaagggaaagagtaagaagctcaagtctgttaaggaacttctcggaatcactatcatggaaaggtcatctttcgagaagaacccaatcgatttcctcgaggctaagggatacaaagaggttaagaaggatctcatcatcaagctcccaaagtactcactcttcgaactcgagaacggtagaaagaggatgctcgcttctgctggtgagcttcaaaagggaaacgagcttgctctcccatctaagtacgttaactttctttacctcgcttctcactacgagaagttgaagggatctccagaagataacgagcagaagcaacttttcgttgagcagcacaagcactacttggatgagatcatcgagcagatctctgagttctctaaaagggtgatcctcgctgatgcaaacctcgataaggtgttgtctgcttacaacaagcacagagataagcctatcagggaacaggcagagaacatcatccatctcttcacccttaccaacctcggtgctcctgctgctttcaagtacttcgatacaaccatcgataggaagagatacacctctaccaaagaagtgctcgatgctaccctcatccatcagtctatcactggactctacgagactaggatcgatctctcacagctcggtggtgattcaagggctgatcctaagaagaagaggaaggttggaggacgccggcggtttgactttaatgggaatgatgaagaagatcttccctttaagaaaggagacatcctgagaatccgggataagcctgaagagcagtggtggaatgcagaggacagcgaaggaaagagggggatgattcttgtcccttacgtggagaagtatgccatggatgctagtgggcaaactacgatcgaagacttctttggtacaaagaaaagcactaatgaggcgcccaataagaaaggtaaatcgggcgctactttcatgaccataacaaatggcgcagctatcaagacagagacaaaggcggtcgcaaaggaggcaaacacggacaaatatcctgctaattcaaatgcaaaagatgtatattcgaagaacttgagcagcaatttacgtacactactgtcgctggagctagaaacgattgatgattcgtggtttccacatttaatggatgaatttaaaaagccatattttgtaaagttgaaacagtttgtcactaaagagcaagctgatcatacagtatttccgcctgcaaaggatatttactcatggaccaggctaacgccttttaataaagttaaagtcgtgattatcggtcaagatccctaccacaactttaatcaggcgcatggcttggcttttagcgtcaaaccccctacaccagcaccaccgtcattaaagaacatatataaggaactgaagcaagagtatcctgattttgttgaagataataaagtgggagatttaactcactgggcttcacaaggggttttattgcttgatacctcgttaactgtaagagcacataatgcaaactcgcattctaagcatggttgggaaacttttacaaaaagggtagttcagttgttgatccaggacagagaggccgacggtaagagtttagtattcctcttatgggggaacaatgctatcaaattagtagagtctctgttgggatctacttccgttggaagcggtagtaagtaccctaatatcatggtgatgaagtcagtgcatccgtctccattaagtgcaagttgtggattttttggtaccaaccatttcaaaatgataaacgattggctatacaatacccgcggagagaaaatgatagactggagtgttgttcctggaacgtcattaagagaagttcaggaggcaaatgctcgcttagagtcagaatcaaaggaccctcctaagaagaaacgtaaagta

SEQ ID NO: 8 - DNA, 6543 bp, Artificial Sequence
  dCas9-UNG1 expression unit (d2)
atggctcctaagaagaagcggaaggttggtattcacggggtgcctgcggctatggataagaagtactctatcggactcgctatcggaactaactctgtgggatgggctgtgatcaccgatgagtacaaggtgccatctaagaagttcaaggttctcggaaacaccgataggcactctatcaagaaaaaccttatcggtgctctcctcttcgattctggtgaaactgctgaggctaccagactcaagagaaccgctagaagaaggtacaccagaagaaagaacaggatctgctacctccaagagatcttctctaacgagatggctaaagtggatgattcattcttccacaggctcgaagagtcattcctcgtggaagaagataagaagcacgagaggcaccctatcttcggaaacatcgttgatgaggtggcataccacgagaagtaccctactatctaccacctcagaaagaagctcgttgattctactgataaggctgatctcaggctcatctacctcgctctcgctcacatgatcaagttcagaggacacttcctcatcgagggtgatctcaaccctgataactctgatgtggataagttgttcatccagctcgtgcagacctacaaccagcttttcgaagagaaccctatcaacgcttcaggtgtggatgctaaggctatcctctctgctaggctctctaagtcaagaaggcttgagaacctcattgctcagctccctggtgagaagaagaacggacttttcggaaacttgatcgctctctctctcggactcacccctaacttcaagtctaacttcgatctcgctgaggatgcaaagctccagctctcaaaggatacctacgatgatgatctcgataacctcctcgctcagatcggagatcagtacgctgatttgttcctcgctgctaagaacctctctgatgctatcctcctcagtgatatcctcagagtgaacaccgagatcaccaaggctccactctcagcttctatgatcaagagatacgatgagcaccaccaggatctcacacttctcaaggctcttgttagacagcagctcccagagaagtacaaagagattttcttcgatcagtctaagaacggatacgctggttacatcgatggtggtgcatctcaagaagagttctacaagttcatcaagcctatcctcgagaagatggatggaaccgaggaactcctcgtgaagctcaatagagaggatcttctcagaaagcagaggaccttcgataacggatctatccctcatcagatccacctcggagagttgcacgctatccttagaaggcaagaggatttctacccattcctcaaggataacagggaaaagattgagaagattctcaccttcagaatcccttactacgtgggacctctcgctagaggaaactcaagattcgcttggatgaccagaaagtctgaggaaaccatcaccccttggaacttcgaagaggtggtggataagggtgctagtgctcagtctttcatcgagaggatgaccaacttcgataagaaccttccaaacgagaaggtgctccctaagcactctttgctctacgagtacttcaccgtgtacaacgagttgaccaaggttaagtacgtgaccgagggaatgaggaagcctgcttttttgtcaggtgagcaaaagaaggctatcgttgatctcttgttcaagaccaacagaaaggtgaccgtgaagcagctcaaagaggattacttcaagaaaatcgagtgcttcgattcagttgagatttctggtgttgaggataggttcaacgcatctctcggaacctaccacgatctcctcaagatcattaaggataaggatttcttggataacgaggaaaacgaggatatcttggaggatatcgttcttaccctcaccctctttgaagatagagagatgattgaagaaaggctcaagacctacgctcatctcttcgatgataaggtgatgaagcagttgaagagaagaagatacactggttggggaaggctctcaagaaagctcattaacggaatcagggataagcagtctggaaagacaatccttgatttcctcaagtctgatggattcgctaacagaaacttcatgcagctcatccacgatgattctctcacctttaaagaggatatccagaaggctcaggtttcaggacagggtgatagtctccatgagcatatcgctaacctcgctggatctcctgcaatcaagaagggaatcctccagactgtgaaggttgtggatgagttggtgaaggtgatgggaaggcataagcctgagaacatcgtgatcgaaatggctagagagaaccagaccactcagaagggacagaagaactctagggaaaggatgaagaggatcgaggaaggtatcaaagagcttggatctcagatcctcaaagagcaccctgttgagaacactcagctccagaatgagaagctctacctctactacctccagaacggaagggatatgtatgtggatcaagagttggatatcaacaggctctctgattacgatgttgatgctatcgtgccacagtcattcttgaaggatgattctatcgataacaaggtgctcaccaggtctgataagaacaggggtaagagtgataacgtgccaagtgaagaggttgtgaagaaaatgaagaactattggaggcagctcctcaacgctaagctcatcactcagagaaagttcgataacttgactaaggctgagaggggaggactctctgaattggataaggcaggattcatcaagaggcagcttgtggaaaccaggcagatcactaagcacgttgcacagatcctcgattctaggatgaacaccaagtacgatgagaacgataagttgatcagggaagtgaaggttatcaccctcaagtcaaagctcgtgtctgatttcagaaaggatttccaattctacaaggtgagggaaatcaacaactaccaccacgctcacgatgcttaccttaacgctgttgttggaaccgctctcatcaagaagtatcctaagctcgagtcagagttcgtgtacggtgattacaaggtgtacgatgtgaggaagatgatcgctaagtctgagcaagagatcggaaaggctaccgctaagtatttcttctactctaacatcatgaatttcttcaagaccgagattaccctcgctaacggtgagatcagaaagaggccactcatcgagacaaacggtgaaacaggtgagatcgtgtgggataagggaagggatttcgctaccgttagaaaggtgctctctatgccacaggtgaacatcgttaagaaaaccgaggtgcagaccggtggattctctaaagagtctatcctccctaagaggaactctgataagctcattgctaggaagaaggattgggaccctaagaaatacggtggtttcgattctcctaccgtggcttactctgttctcgttgtggctaaggttgagaagggaaagagtaagaagctcaagtctgttaaggaacttctcggaatcactatcatggaaaggtcatctttcgagaagaacccaatcgatttcctcgaggctaagggatacaaagaggttaagaaggatctcatcatcaagctcccaaagtactcactcttcgaactcgagaacggtagaaagaggatgctcgcttctgctggtgagcttcaaaagggaaacgagcttgctctcccatctaagtacgttaactttctttacctcgcttctcactacgagaagttgaagggatctccagaagataacgagcagaagcaacttttcgttgagcagcacaagcactacttggatgagatcatcgagcagatctctgagttctctaaaagggtgatcctcgctgatgcaaacctcgataaggtgttgtctgcttacaacaagcacagagataagcctatcagggaacaggcagagaacatcatccatctcttcacccttaccaacctcggtgctcctgctgctttcaagtacttcgatacaaccatcgataggaagagatacacctctaccaaagaagtgctcgatgctaccctcatccatcagtctatcactggactctacgagactaggatcgatctctcacagctcggtggtgattcaagggctgatcctaagaagaagaggaaggttggaggacgccggcggtttgactttaatgggaatgatgaagaagatcttccctttaagaaaggagacatcctgagaatccgggataagcctgaagagcagtggtggaatgcagaggacagcgaaggaaagagggggatgattcttgtcccttacgtggagaagtatgccatggatgctagtgggcaaactacgatcgaagacttctttggtacaaagaaaagcactaatgaggcgcccaataagaaaggtaaatcgggcgctactttcatgaccataacaaatggcgcagctatcaagacagagacaaaggcggtcgcaaaggaggcaaacacggacaaatatcctgctaattcaaatgcaaaagatgtatattcgaagaacttgagcagcaatttacgtacactactgtcgctggagctagaaacgattgatgattcgtggtttccacatttaatggatgaatttaaaaagccatattttgtaaagttgaaacagtttgtcactaaagagcaagctgatcatacagtatttccgcctgcaaaggatatttactcatggaccaggctaacgccttttaataaagttaaagtcgtgattatcggtcaagatccctaccacaactttaatcaggcgcatggcttggcttttagcgtcaaaccccctacaccagcaccaccgtcattaaagaacatatataaggaactgaagcaagagtatcctgattttgttgaagataataaagtgggagatttaactcactgggcttcacaaggggttttattgcttgatacctcgttaactgtaagagcacataatgcaaactcgcattctaagcatggttgggaaacttttacaaaaagggtagttcagttgttgatccaggacagagaggccgacggtaagagtttagtattcctcttatgggggaacaatgctatcaaattagtagagtctctgttgggatctacttccgttggaagcggtagtaagtaccctaatatcatggtgatgaagtcagtgcatccgtctccattaagtgcaagttgtggattttttggtaccaaccatttcaaaatgataaacgattggctatacaatacccgcggagagaaaatgatagactggagtgttgttcctggaacgtcattaagagaagttcaggaggcaaatgctcgcttagagtcagaatcaaaggaccctactagaggctccggaggtggcggcgcgtcgacgtccggagactataaggaccacgacggagactacaaggatcatgatattgattacaaagacgatgacgataagtctagcaaaatgcaaactacgatcgaagacttctttggtacaaagaaaagcactaatgaggcgcccaataagaaaggtaaatcgggcgctactttcatgaccataacaaatggcgcagctatcaagacagagacaaaggcggtcgcaaaggaggcaaacacggacaaatatcctgctaattcaaatgcaaaagatgtatattcgaagaacttgagcagcaatttacgtacactactgtcgctggagctagaaacgattgatgattcgtggtttccacatttaatggatgaatttaaaaagccatattttgtaaagttgaaacagtttgtcactaaagagcaagctgatcatacagtatttccgcctgcaaaggatatttactcatggaccaggctaacgccttttaataaagttaaagtcgtgattatcggtcaagatccctaccacaactttaatcaggcgcatggcttggcttttagcgtcaaaccccctacaccagcaccaccgtcattaaagaacatatataaggaactgaagcaagagtatcctgattttgttgaagataataaagtgggagatttaactcactgggcttcacaaggggttttattgcttgatacctcgttaactgtaagagcacataatgcaaactcgcattctaagcatggttgggaaacttttacaaaaagggtagttcagttgttgatccaggacagagaggccgacggtaagagtttagtattcctcttatgggggaacaatgctatcaaattagtagagtctctgttgggatctacttccgttggaagcggtagtaagtaccctaatatcatggtgatgaagtcagtgcatccgtctccattaagtgcaagttgtggattttttggtaccaaccatttcaaaatgataaacgattggctatacaatacccgcggagagaaaatgatagactggagtgttgttcctggaacgtcattaagagaagttcaggaggcaaatgctcgcttagagtcagaatcaaaggaccctcctaagaagaaacgtaaagta

SEQ ID NO: 9 - DNA, 5358 bp, Artificial Sequence
  nCas9-UNG1 expression unit (n1)
atggataagaagtactctatcggactcgctatcggaactaactctgtgggatgggctgtgatcaccgatgagtacaaggtgccatctaagaagttcaaggttctcggaaacaccgataggcactctatcaagaaaaaccttatcggtgctctcctcttcgattctggtgaaactgctgaggctaccagactcaagagaaccgctagaagaaggtacaccagaagaaagaacaggatctgctacctccaagagatcttctctaacgagatggctaaagtggatgattcattcttccacaggctcgaagagtcattcctcgtggaagaagataagaagcacgagaggcaccctatcttcggaaacatcgttgatgaggtggcataccacgagaagtaccctactatctaccacctcagaaagaagctcgttgattctactgataaggctgatctcaggctcatctacctcgctctcgctcacatgatcaagttcagaggacacttcctcatcgagggtgatctcaaccctgataactctgatgtggataagttgttcatccagctcgtgcagacctacaaccagcttttcgaagagaaccctatcaacgcttcaggtgtggatgctaaggctatcctctctgctaggctctctaagtcaagaaggcttgagaacctcattgctcagctccctggtgagaagaagaacggacttttcggaaacttgatcgctctctctctcggactcacccctaacttcaagtctaacttcgatctcgctgaggatgcaaagctccagctctcaaaggatacctacgatgatgatctcgataacctcctcgctcagatcggagatcagtacgctgatttgttcctcgctgctaagaacctctctgatgctatcctcctcagtgatatcctcagagtgaacaccgagatcaccaaggctccactctcagcttctatgatcaagagatacgatgagcaccaccaggatctcacacttctcaaggctcttgttagacagcagctcccagagaagtacaaagagattttcttcgatcagtctaagaacggatacgctggttacatcgatggtggtgcatctcaagaagagttctacaagttcatcaagcctatcctcgagaagatggatggaaccgaggaactcctcgtgaagctcaatagagaggatcttctcagaaagcagaggaccttcgataacggatctatccctcatcagatccacctcggagagttgcacgctatccttagaaggcaagaggatttctacccattcctcaaggataacagggaaaagattgagaagattctcaccttcagaatcccttactacgtgggacctctcgctagaggaaactcaagattcgcttggatgaccagaaagtctgaggaaaccatcaccccttggaacttcgaagaggtggtggataagggtgctagtgctcagtctttcatcgagaggatgaccaacttcgataagaaccttccaaacgagaaggtgctccctaagcactctttgctctacgagtacttcaccgtgtacaacgagttgaccaaggttaagtacgtgaccgagggaatgaggaagcctgcttttttgtcaggtgagcaaaagaaggctatcgttgatctcttgttcaagaccaacagaaaggtgaccgtgaagcagctcaaagaggattacttcaagaaaatcgagtgcttcgattcagttgagatttctggtgttgaggataggttcaacgcatctctcggaacctaccacgatctcctcaagatcattaaggataaggatttcttggataacgaggaaaacgaggatatcttggaggatatcgttcttaccctcaccctctttgaagatagagagatgattgaagaaaggctcaagacctacgctcatctcttcgatgataaggtgatgaagcagttgaagagaagaagatacactggttggggaaggctctcaagaaagctcattaacggaatcagggataagcagtctggaaagacaatccttgatttcctcaagtctgatggattcgctaacagaaacttcatgcagctcatccacgatgattctctcacctttaaagaggatatccagaaggctcaggtttcaggacagggtgatagtctccatgagcatatcgctaacctcgctggatctcctgcaatcaagaagggaatcctccagactgtgaaggttgtggatgagttggtgaaggtgatgggaaggcataagcctgagaacatcgtgatcgaaatggctagagagaaccagaccactcagaagggacagaagaactctagggaaaggatgaagaggatcgaggaaggtatcaaagagcttggatctcagatcctcaaagagcaccctgttgagaacactcagctccagaatgagaagctctacctctactacctccagaacggaagggatatgtatgtggatcaagagttggatatcaacaggctctctgattacgatgttgatgctatcgtgccacagtcattcttgaaggatgattctatcgataacaaggtgctcaccaggtctgataagaacaggggtaagagtgataacgtgccaagtgaagaggttgtgaagaaaatgaagaactattggaggcagctcctcaacgctaagctcatcactcagagaaagttcgataacttgactaaggctgagaggggaggactctctgaattggataaggcaggattcatcaagaggcagcttgtggaaaccaggcagatcactaagcacgttgcacagatcctcgattctaggatgaacaccaagtacgatgagaacgataagttgatcagggaagtgaaggttatcaccctcaagtcaaagctcgtgtctgatttcagaaaggatttccaattctacaaggtgagggaaatcaacaactaccaccacgctcacgatgcttaccttaacgctgttgttggaaccgctctcatcaagaagtatcctaagctcgagtcagagttcgtgtacggtgattacaaggtgtacgatgtgaggaagatgatcgctaagtctgagcaagagatcggaaaggctaccgctaagtatttcttctactctaacatcatgaatttcttcaagaccgagattaccctcgctaacggtgagatcagaaagaggccactcatcgagacaaacggtgaaacaggtgagatcgtgtgggataagggaagggatttcgctaccgttagaaaggtgctctctatgccacaggtgaacatcgttaagaaaaccgaggtgcagaccggtggattctctaaagagtctatcctccctaagaggaactctgataagctcattgctaggaagaaggattgggaccctaagaaatacggtggtttcgattctcctaccgtggcttactctgttctcgttgtggctaaggttgagaagggaaagagtaagaagctcaagtctgttaaggaacttctcggaatcactatcatggaaaggtcatctttcgagaagaacccaatcgatttcctcgaggctaagggatacaaagaggttaagaaggatctcatcatcaagctcccaaagtactcactcttcgaactcgagaacggtagaaagaggatgctcgcttctgctggtgagcttcaaaagggaaacgagcttgctctcccatctaagtacgttaactttctttacctcgcttctcactacgagaagttgaagggatctccagaagataacgagcagaagcaacttttcgttgagcagcacaagcactacttggatgagatcatcgagcagatctctgagttctctaaaagggtgatcctcgctgatgcaaacctcgataaggtgttgtctgcttacaacaagcacagagataagcctatcagggaacaggcagagaacatcatccatctcttcacccttaccaacctcggtgctcctgctgctttcaagtacttcgatacaaccatcgataggaagagatacacctctaccaaagaagtgctcgatgctaccctcatccatcagtctatcactggactctacgagactaggatcgatctctcacagctcggtggtgattcaagggctgatcctaagaagaagaggaaggttggaggacgccggcggtttgactttaatgggaatgatgaagaagatcttccctttaagaaaggagacatcctgagaatccgggataagcctgaagagcagtggtggaatgcagaggacagcgaaggaaagagggggatgattcttgtcccttacgtggagaagtatgccatggatgctagtgggcaaactacgatcgaagacttctttggtacaaagaaaagcactaatgaggcgcccaataagaaaggtaaatcgggcgctactttcatgaccataacaaatggcgcagctatcaagacagagacaaaggcggtcgcaaaggaggcaaacacggacaaatatcctgctaattcaaatgcaaaagatgtatattcgaagaacttgagcagcaatttacgtacactactgtcgctggagctagaaacgattgatgattcgtggtttccacatttaatggatgaatttaaaaagccatattttgtaaagttgaaacagtttgtcactaaagagcaagctgatcatacagtatttccgcctgcaaaggatatttactcatggaccaggctaacgccttttaataaagttaaagtcgtgattatcggtcaagatccctaccacaactttaatcaggcgcatggcttggcttttagcgtcaaaccccctacaccagcaccaccgtcattaaagaacatatataaggaactgaagcaagagtatcctgattttgttgaagataataaagtgggagatttaactcactgggcttcacaaggggttttattgcttgatacctcgttaactgtaagagcacataatgcaaactcgcattctaagcatggttgggaaacttttacaaaaagggtagttcagttgttgatccaggacagagaggccgacggtaagagtttagtattcctcttatgggggaacaatgctatcaaattagtagagtctctgttgggatctacttccgttggaagcggtagtaagtaccctaatatcatggtgatgaagtcagtgcatccgtctccattaagtgcaagttgtggattttttggtaccaaccatttcaaaatgataaacgattggctatacaatacccgcggagagaaaatgatagactggagtgttgttcctggaacgtcattaagagaagttcaggaggcaaatgctcgcttagagtcagaatcaaaggaccctcctaagaagaaacgtaaagta

SEQ ID NO: 10 - DNA, 6492 bp, Artificial Sequence
  nCas9-UNG1 expression unit (n2)
atggataagaagtactctatcggactcgctatcggaactaactctgtgggatgggctgtgatcaccgatgagtacaaggtgccatctaagaagttcaaggttctcggaaacaccgataggcactctatcaagaaaaaccttatcggtgctctcctcttcgattctggtgaaactgctgaggctaccagactcaagagaaccgctagaagaaggtacaccagaagaaagaacaggatctgctacctccaagagatcttctctaacgagatggctaaagtggatgattcattcttccacaggctcgaagagtcattcctcgtggaagaagataagaagcacgagaggcaccctatcttcggaaacatcgttgatgaggtggcataccacgagaagtaccctactatctaccacctcagaaagaagctcgttgattctactgataaggctgatctcaggctcatctacctcgctctcgctcacatgatcaagttcagaggacacttcctcatcgagggtgatctcaaccctgataactctgatgtggataagttgttcatccagctcgtgcagacctacaaccagcttttcgaagagaaccctatcaacgcttcaggtgtggatgctaaggctatcctctctgctaggctctctaagtcaagaaggcttgagaacctcattgctcagctccctggtgagaagaagaacggacttttcggaaacttgatcgctctctctctcggactcacccctaacttcaagtctaacttcgatctcgctgaggatgcaaagctccagctctcaaaggatacctacgatgatgatctcgataacctcctcgctcagatcggagatcagtacgctgatttgttcctcgctgctaagaacctctctgatgctatcctcctcagtgatatcctcagagtgaacaccgagatcaccaaggctccactctcagcttctatgatcaagagatacgatgagcaccaccaggatctcacacttctcaaggctcttgttagacagcagctcccagagaagtacaaagagattttcttcgatcagtctaagaacggatacgctggttacatcgatggtggtgcatctcaagaagagttctacaagttcatcaagcctatcctcgagaagatggatggaaccgaggaactcctcgtgaagctcaatagagaggatcttctcagaaagcagaggaccttcgataacggatctatccctcatcagatccacctcggagagttgcacgctatccttagaaggcaagaggatttctacccattcctcaaggataacagggaaaagattgagaagattctcaccttcagaatcccttactacgtgggacctctcgctagaggaaactcaagattcgcttggatgaccagaaagtctgaggaaaccatcaccccttggaacttcgaagaggtggtggataagggtgctagtgctcagtctttcatcgagaggatgaccaacttcgataagaaccttccaaacgagaaggtgctccctaagcactctttgctctacgagtacttcaccgtgtacaacgagttgaccaaggttaagtacgtgaccgagggaatgaggaagcctgcttttttgtcaggtgagcaaaagaaggctatcgttgatctcttgttcaagaccaacagaaaggtgaccgtgaagcagctcaaagaggattacttcaagaaaatcgagtgcttcgattcagttgagatttctggtgttgaggataggttcaacgcatctctcggaacctaccacgatctcctcaagatcattaaggataaggatttcttggataacgaggaaaacgaggatatcttggaggatatcgttcttaccctcaccctctttgaagatagagagatgattgaagaaaggctcaagacctacgctcatctcttcgatgataaggtgatgaagcagttgaagagaagaagatacactggttggggaaggctctcaagaaagctcattaacggaatcagggataagcagtctggaaagacaatccttgatttcctcaagtctgatggattcgctaacagaaacttcatgcagctcatccacgatgattctctcacctttaaagaggatatccagaaggctcaggtttcaggacagggtgatagtctccatgagcatatcgctaacctcgctggatctcctgcaatcaagaagggaatcctccagactgtgaaggttgtggatgagttggtgaaggtgatgggaaggcataagcctgagaacatcgtgatcgaaatggctagagagaaccagaccactcagaagggacagaagaactctagggaaaggatgaagaggatcgaggaaggtatcaaagagcttggatctcagatcctcaaagagcaccctgttgagaacactcagctccagaatgagaagctctacctctactacctccagaacggaagggatatgtatgtggatcaagagttggatatcaacaggctctctgattacgatgttgatgctatcgtgccacagtcattcttgaaggatgattctatcgataacaaggtgctcaccaggtctgataagaacaggggtaagagtgataacgtgccaagtgaagaggttgtgaagaaaatgaagaactattggaggcagctcctcaacgctaagctcatcactcagagaaagttcgataacttgactaaggctgagaggggaggactctctgaattggataaggcaggattcatcaagaggcagcttgtggaaaccaggcagatcactaagcacgttgcacagatcctcgattctaggatgaacaccaagtacgatgagaacgataagttgatcagggaagtgaaggttatcaccctcaagtcaaagctcgtgtctgatttcagaaaggatttccaattctacaaggtgagggaaatcaacaactaccaccacgctcacgatgcttaccttaacgctgttgttggaaccgctctcatcaagaagtatcctaagctcgagtcagagttcgtgtacggtgattacaaggtgtacgatgtgaggaagatgatcgctaagtctgagcaagagatcggaaaggctaccgctaagtatttcttctactctaacatcatgaatttcttcaagaccgagattaccctcgctaacggtgagatcagaaagaggccactcatcgagacaaacggtgaaacaggtgagatcgtgtgggataagggaagggatttcgctaccgttagaaaggtgctctctatgccacaggtgaacatcgttaagaaaaccgaggtgcagaccggtggattctctaaagagtctatcctccctaagaggaactctgataagctcattgctaggaagaaggattgggaccctaagaaatacggtggtttcgattctcctaccgtggcttactctgttctcgttgtggctaaggttgagaagggaaagagtaagaagctcaagtctgttaaggaacttctcggaatcactatcatggaaaggtcatctttcgagaagaacccaatcgatttcctcgaggctaagggatacaaagaggttaagaaggatctcatcatcaagctcccaaagtactcactcttcgaactcgagaacggtagaaagaggatgctcgcttctgctggtgagcttcaaaagggaaacgagcttgctctcccatctaagtacgttaactttctttacctcgcttctcactacgagaagttgaagggatctccagaagataacgagcagaagcaacttttcgttgagcagcacaagcactacttggatgagatcatcgagcagatctctgagttctctaaaagggtgatcctcgctgatgcaaacctcgataaggtgttgtctgcttacaacaagcacagagataagcctatcagggaacaggcagagaacatcatccatctcttcacccttaccaacctcggtgctcctgctgctttcaagtacttcgatacaaccatcgataggaagagatacacctctaccaaagaagtgctcgatgctaccctcatccatcagtctatcactggactctacgagactaggatcgatctctcacagctcggtggtgattcaagggctgatcctaagaagaagaggaaggttggaggacgccggcggtttgactttaatgggaatgatgaagaagatcttccctttaagaaaggagacatcctgagaatccgggataagcctgaagagcagtggtggaatgcagaggacagcgaaggaaagagggggatgattcttgtcccttacgtggagaagtatgccatggatgctagtgggcaaactacgatcgaagacttctttggtacaaagaaaagcactaatgaggcgcccaataagaaaggtaaatcgggcgctactttcatgaccataacaaatggcgcagctatcaagacagagacaaaggcggtcgcaaaggaggcaaacacggacaaatatcctgctaattcaaatgcaaaagatgtatattcgaagaacttgagcagcaatttacgtacactactgtcgctggagctagaaacgattgatgattcgtggtttccacatttaatggatgaatttaaaaagccatattttgtaaagttgaaacagtttgtcactaaagagcaagctgatcatacagtatttccgcctgcaaaggatatttactcatggaccaggctaacgccttttaataaagttaaagtcgtgattatcggtcaagatccctaccacaactttaatcaggcgcatggcttggcttttagcgtcaaaccccctacaccagcaccaccgtcattaaagaacatatataaggaactgaagcaagagtatcctgattttgttgaagataataaagtgggagatttaactcactgggcttcacaaggggttttattgcttgatacctcgttaactgtaagagcacataatgcaaactcgcattctaagcatggttgggaaacttttacaaaaagggtagttcagttgttgatccaggacagagaggccgacggtaagagtttagtattcctcttatgggggaacaatgctatcaaattagtagagtctctgttgggatctacttccgttggaagcggtagtaagtaccctaatatcatggtgatgaagtcagtgcatccgtctccattaagtgcaagttgtggattttttggtaccaaccatttcaaaatgataaacgattggctatacaatacccgcggagagaaaatgatagactggagtgttgttcctggaacgtcattaagagaagttcaggaggcaaatgctcgcttagagtcagaatcaaaggaccctactagaggctccggaggtggcggcgcgtcgacgtccggagactataaggaccacgacggagactacaaggatcatgatattgattacaaagacgatgacgataagtctagcaaaatgcaaactacgatcgaagacttctttggtacaaagaaaagcactaatgaggcgcccaataagaaaggtaaatcgggcgctactttcatgaccataacaaatggcgcagctatcaagacagagacaaaggcggtcgcaaaggaggcaaacacggacaaatatcctgctaattcaaatgcaaaagatgtatattcgaagaacttgagcagcaatttacgtacactactgtcgctggagctagaaacgattgatgattcgtggtttccacatttaatggatgaatttaaaaagccatattttgtaaagttgaaacagtttgtcactaaagagcaagctgatcatacagtatttccgcctgcaaaggatatttactcatggaccaggctaacgccttttaataaagttaaagtcgtgattatcggtcaagatccctaccacaactttaatcaggcgcatggcttggcttttagcgtcaaaccccctacaccagcaccaccgtcattaaagaacatatataaggaactgaagcaagagtatcctgattttgttgaagataataaagtgggagatttaactcactgggcttcacaaggggttttattgcttgatacctcgttaactgtaagagcacataatgcaaactcgcattctaagcatggttgggaaacttttacaaaaagggtagttcagttgttgatccaggacagagaggccgacggtaagagtttagtattcctcttatgggggaacaatgctatcaaattagtagagtctctgttgggatctacttccgttggaagcggtagtaagtaccctaatatcatggtgatgaagtcagtgcatccgtctccattaagtgcaagttgtggattttttggtaccaaccatttcaaaatgataaacgattggctatacaatacccgcggagagaaaatgatagactggagtgttgttcctggaacgtcattaagagaagttcaggaggcaaatgctcgcttagagtcagaatcaaaggaccctcctaagaagaaacgtaaagta

SEQ ID NO: 11 - DNA, 247 bp, Oryza sativa
ggatcatgaaccaacggcctggctgtatttggtggttgtgtagggagatggggagaagaaaagcccgattctcttcgctgtgatgggctggatgcatgcgggggagcgggaggcccaagtacgtgcacggtgagcggcccacagggcgagtgtgagcgcgagaggcgggaggaacagtttagtaccacattgcccagctaactcgaacgcgaccaacttataaacccgcgcgctgtcgcttgtgttg

SEQ ID NO: 12 - DNA, 20 bp, Artificial Sequence
  guide RNA: ALS A96
catggacgcgccgcccgggt

SEQ ID NO: 13 - DNA, 20 bp, Artificial Sequence
  guide RNA: OsFTIP1e Q590
cagctgtggaaaccaccaat

SEQ ID NO: 14 - DNA, 20 bp, Artificial Sequence
  guide RNA: DL-3
gaccttgcactgactgcagg

SEQ ID NO: 15 - DNA, 20 bp, Artificial Sequence
  guide RNA: OsClpP5
gccatggccgcggctcgtgg

SEQ ID NO: 16 - DNA, 20 bp, Artificial Sequence
  guide RNA: EGFP Mut1
gagctggacggcgacgtaaa

SEQ ID NO: 17 - DNA, 20 bp, Artificial Sequence
  guide RNA: EGFP Mut2
catgtgatcgcgcttctcgt

SEQ ID NO: 18 - DNA, 20 bp, Artificial Sequence
  guide RNA: mGFP switch
tctagaggatccggcccagt

SEQ ID NO: 19 - DNA, 20 bp, Artificial Sequence
  guide RNA: ALS P171-R173
caggtcccccgccgcatgat

SEQ ID NO: 20 - DNA, 1173 bp, Artificial Sequence
  guide RNA unit x4
ggatcatgaaccaacggcctggctgtatttggtggttgtgtagggagatggggagaagaaaagcccgattctcttcgctgtgatgggctggatgcatgcgggggagcgggaggcccaagtacgtgcacggtgagcggcccacagggcgagtgtgagcgcgagaggcgggaggaacagtttagtaccacattgcccagctaactcgaacgcgaccaacttataaacccgcgcgctgtcgcttgtgttgcgcgtccatggagatccaccgttttagagctagaaatagcaagttaaaataaggctagtccgttatcaacttgaaaaagtggcaccgagtcggtgctttttttgtcccttcgaagggcaattctgcatctagcccagtgtgctggaattgcccttggatcatgaaccaacggcctggctgtatttggtggttgtgtagggagatggggagaagaaaagcccgattctcttcgctgtgatgggctggatgcatgcgggggagcgggaggcccaagtacgtgcacggtgagcggcccacagggcgagtgtgagcgcgagaggcgggaggaacagtttagtaccacattgcccagctaactcgaacgcgaccaacttataaacccgcgcgctgtcgcttgtgttggaccttgcactgactgcagggttttagagctagaaatagcaagttaaaataaggctagtccgttatcaacttgaaaaagtggcaccgagtcggtgctttttttgtcccttcgaagggcaattctgcatctagcccagtgtgctggaattgcccttggatcatgaaccaacggcctggctgtatttggtggttgtgtagggagatggggagaagaaaagcccgattctcttcgctgtgatgggctggatgcatgcgggggagcgggaggcccaagtacgtgcacggtgagcggcccacagggcgagtgtgagcgcgagaggcgggaggaacagtttagtaccacattgcccagctaactcgaacgcgaccaacttataaacccgcgcgctgtcgcttgtgttgcagctgtggaaaccaccaatgttttagagctagaaatagcaagttaaaataaggctagtccgttatcaacttgaaaaagtggcaccgagtcggtgctttttttgtcccttcgaagggcaatt

SEQ ID NO: 21 - DNA, 2379 bp, Artificial Sequence
  guide RNA unit x6
ggatcatgaaccaacggcctggctgtatttggtggttgtgtagggagatggggagaagaaaagcccgattctcttcgctgtgatgggctggatgcatgcgggggagcgggaggcccaagtacgtgcacggtgagcggcccacagggcgagtgtgagcgcgagaggcgggaggaacagtttagtaccacattgcccagctaactcgaacgcgaccaacttataaacccgcgcgctgtcgcttgtgttgcgcgtccatggagatccaccgttttagagctagaaatagcaagttaaaataaggctagtccgttatcaacttgaaaaagtggcaccgagtcggtgctttttttgtcccttcgaagggcaattctgcatctagcccagtgtgctggaattgcccttggatcatgaaccaacggcctggctgtatttggtggttgtgtagggagatggggagaagaaaagcccgattctcttcgctgtgatgggctggatgcatgcgggggagcgggaggcccaagtacgtgcacggtgagcggcccacagggcgagtgtgagcgcgagaggcgggaggaacagtttagtaccacattgcccagctaactcgaacgcgaccaacttataaacccgcgcgctgtcgcttgtgttggaccttgcactgactgcagggttttagagctagaaatagcaagttaaaataaggctagtccgttatcaacttgaaaaagtggcaccgagtcggtgctttttttgtcccttcgaagggcaattctgcatctagcccagtgtgctggaattgcccttggatcatgaaccaacggcctggctgtatttggtggttgtgtagggagatggggagaagaaaagcccgattctcttcgctgtgatgggctggatgcatgcgggggagcgggaggcccaagtacgtgcacggtgagcggcccacagggcgagtgtgagcgcgagaggcgggaggaacagtttagtaccacattgcccagctaactcgaacgcgaccaacttataaacccgcgcgctgtcgcttgtgttgcagctgtggaaaccaccaatgttttagagctagaaatagcaagttaaaataaggctagtccgttatcaacttgaaaaagtggcaccgagtcggtgctttttttgtcccttcgaagggcaattctgcatctagcccagtgtgctggaattgcccttggatcatgaaccaacggcctggctgtatttggtggttgtgtagggagatggggagaagaaaagcccgattctcttcgctgtgatgggctggatgcatgcgggggagcgggaggcccaagtacgtgcacggtgagcggcccacagggcgagtgtgagcgcgagaggcgggaggaacagtttagtaccacattgcccagctaactcgaacgcgaccaacttataaacccgcgcgctgtcgcttgtgttggccatggccgcggctcgtgggttttagagctagaaatagcaagttaaaataaggctagtccgttatcaacttgaaaaagtggcaccgagtcggtgctttttttgtcccttcgaagggcaattctgcatctagcccagtgtgctggaattgcccttggatcatgaaccaacggcctggctgtatttggtggttgtgtagggagatggggagaagaaaagcccgattctcttcgctgtgatgggctggatgcatgcgggggagcgggaggcccaagtacgtgcacggtgagcggcccacagggcgagtgtgagcgcgagaggcgggaggaacagtttagtaccacattgcccagctaactcgaacgcgaccaacttataaacccgcgcgctgtcgcttgtgttggagctggacggcgacgtaaagttttagagctagaaatagcaagttaaaataaggctagtccgttatcaacttgaaaaagtggcaccgagtcggtgctttttttgtcccttcgaagggcaattctgcatctagcccagtgtgctggaattgcccttggatcatgaaccaacggcctggctgtatttggtggttgtgtagggagatggggagaagaaaagcccgattctcttcgctgtgatgggctggatgcatgcgggggagcgggaggcccaagtacgtgcacggtgagcggcccacagggcgagtgtgagcgcgagaggcgggaggaacagtttagtaccacattgcccagctaactcgaacgcgaccaacttataaacccgcgcgctgtcgcttgtgttgcatgtgatcgcgcttctcgtgttttagagctagaaatagcaagttaaaataaggctagtccgttatcaacttgaaaaagtggcaccgagtcggtgctttttttgtcccttcgaagggcaatt

SEQ ID NO: 22 - DNA, 1977 bp, Artificial Sequence
  guide RNA unit x5
ggatcatgaaccaacggcctggctgtatttggtggttgtgtagggagatggggagaagaaaagcccgattctcttcgctgtgatgggctggatgcatgcgggggagcgggaggcccaagtacgtgcacggtgagcggcccacagggcgagtgtgagcgcgagaggcgggaggaacagtttagtaccacattgcccagctaactcgaacgcgaccaacttataaacccgcgcgctgtcgcttgtgttgcgcgtccatggagatccaccgttttagagctagaaatagcaagttaaaataaggctagtccgttatcaacttgaaaaagtggcaccgagtcggtgctttttttgtcccttcgaagggcaattctgcatctagcccagtgtgctggaattgcccttggatcatgaaccaacggcctggctgtatttggtggttgtgtagggagatggggagaagaaaagcccgattctcttcgctgtgatgggctggatgcatgcgggggagcgggaggcccaagtacgtgcacggtgagcggcccacagggcgagtgtgagcgcgagaggcgggaggaacagtttagtaccacattgcccagctaactcgaacgcgaccaacttataaacccgcgcgctgtcgcttgtgttggaccttgcactgactgcagggttttagagctagaaatagcaagttaaaataaggctagtccgttatcaacttgaaaaagtggcaccgagtcggtgctttttttgtcccttcgaagggcaattctgcatctagcccagtgtgctggaattgcccttggatcatgaaccaacggcctggctgtatttggtggttgtgtagggagatggggagaagaaaagcccgattctcttcgctgtgatgggctggatgcatgcgggggagcgggaggcccaagtacgtgcacggtgagcggcccacagggcgagtgtgagcgcgagaggcgggaggaacagtttagtaccacattgcccagctaactcgaacgcgaccaacttataaacccgcgcgctgtcgcttgtgttgcagctgtggaaaccaccaatgttttagagctagaaatagcaagttaaaataaggctagtccgttatcaacttgaaaaagtggcaccgagtcggtgctttttttgtcccttcgaagggcaattctgcatctagcccagtgtgctggaattgcccttggatcatgaaccaacggcctggctgtatttggtggttgtgtagggagatggggagaagaaaagcccgattctcttcgctgtgatgggctggatgcatgcgggggagcgggaggcccaagtacgtgcacggtgagcggcccacagggcgagtgtgagcgcgagaggcgggaggaacagtttagtaccacattgcccagctaactcgaacgcgaccaacttataaacccgcgcgctgtcgcttgtgttggccatggccgcggctcgtgggttttagagctagaaatagcaagttaaaataaggctagtccgttatcaacttgaaaaagtggcaccgagtcggtgctttttttgtcccttcgaagggcaattctgcatctagcccagtgtgctggaattgcccttggatcatgaaccaacggcctggctgtatttggtggttgtgtagggagatggggagaagaaaagcccgattctcttcgctgtgatgggctggatgcatgcgggggagcgggaggcccaagtacgtgcacggtgagcggcccacagggcgagtgtgagcgcgagaggcgggaggaacagtttagtaccacattgcccagctaactcgaacgcgaccaacttataaacccgcgcgctgtcgcttgtgttgtctagaggatccggcccagtgttttagagctagaaatagcaagttaaaataaggctagtccgttatcaacttgaaaaagtggcaccgagtcggtgctttttttgtcccttcgaagggcaatt

SEQ ID NO: 23 - DNA, 771 bp, Artificial Sequence
  guide RNA unit x2
ggatcatgaaccaacggcctggctgtatttggtggttgtgtagggagatggggagaagaaaagcccgattctcttcgctgtgatgggctggatgcatgcgggggagcgggaggcccaagtacgtgcacggtgagcggcccacagggcgagtgtgagcgcgagaggcgggaggaacagtttagtaccacattgcccagctaactcgaacgcgaccaacttataaacccgcgcgctgtcgcttgtgttgcatggacgcgccgcccgggtgttttagagctagaaatagcaagttaaaataaggctagtccgttatcaacttgaaaaagtggcaccgagtcggtgctttttttgtcccttcgaagggcaattctgcatctagcccagtgtgctggaattgcccttggatcatgaaccaacggcctggctgtatttggtggttgtgtagggagatggggagaagaaaagcccgattctcttcgctgtgatgggctggatgcatgcgggggagcgggaggcccaagtacgtgcacggtgagcggcccacagggcgagtgtgagcgcgagaggcgggaggaacagtttagtaccacattgcccagctaactcgaacgcgaccaacttataaacccgcgcgctgtcgcttgtgttgcaggtcccccgccgcatgatgttttagagctagaaatagcaagttaaaataaggctagtccgttatcaacttgaaaaagtggcaccgagtcggtgctttttttgtcccttcgaagggcaatt

SEQ ID NO: 24 - DNA, 2088 bp, Artificial Sequence
  hygromycin phosphotransferase (hpt) expression unit
agattagccttttcaatttcagaaagaatgctaacccacagatggttagagaggcttacgcagcaggtctcatcaagacgatctacccgagcaataatctccaggaaatcaaataccttcccaagaaggttaaagatgcagtcaaaagattcaggactaactgcatcaagaacacagagaaagatatatttctcaagatcagaagtactattccagtatggacgattcaaggcttgcttcacaaaccaaggcaagtaatagagattggagtctctaaaaaggtagttcccactgaatcaaaggccatggagtcaaagattcaaatagaggacctaacagaactcgccgtaaagactggcgaacagttcatacagagtctcttacgactcaatgacaagaagaaaatcttcgtcaacatggtggagcacgacacacttgtctactccaaaaatatcaaagatacagtctcagaagaccaaagggcaattgagacttttcaacaaagggtaatatccggaaacctcctcggattccattgcccagctatctgtcactttattgtgaagatagtggaaaaggaaggtggctcctacaaatgccatcattgcgataaaggaaaggccatcgttgaagatgcctctgccgacagtggtcccaaagatggacccccacccacgaggagcatcgtggaaaaagaagacgttccaaccacgtcttcaaagcaagtggattgatgtgatatctccactgacgtaagggatgacgcacaatcccactatccttcgcaagacccttcctctatataaggaagttcatttcatttggagagaacacgggggactctagaatgaaaaagcctgaactcaccgccacgtctgtcgagaagtttctgatcgaaaagttcgacagcgtctccgacctgatgcagctctcggagggcgaagaatctcgtgctttcagcttcgatgtaggagggcgtggatatgtcctgcgggtaaatagctgcgccgatggtttctacaaagatcgttatgtttatcggcactttgcatcggccgcgctcccgattccggaagtgcttgacattggggaattcagcgagagcctgacctattgcatctcccgccgtgcacagggtgtcacgttgcaagacctgcctgaaaccgaactgcccgctgttctgcagccggtcgcggaggccatggatgcgatcgctgcggccgatcttagccagacgagcgggttcggcccattcggaccgcaaggaatcggtcaatacactacatggcgtgatttcatatgcgcgattgctgatccccatgtgtatcactggcaaactgtgatggacgacaccgtcagtgcgtccgtcgcgcaggctctcgatgagctgatgctttgggccgaggactgccccgaagtccggcacctcgtgcacgcggatttcggctccaacaatgtcctgacggacaatggccgcataacagcggtcattgactggagcgaggcgatgttcggggattcccaatacgaggtcgccaacatcttcttctggaggccgtggttggcttgtatggagcagcagacgcgctacttcgagcggaggcatccggagcttgcaggatcgccgcggctccgggcgtatatgctccgcattggtcttgaccaactctatcagagcttggttgacggcaatttcgatgatgcagcttgggcgcagggtcgatgcgacgcaatcgtccgatccggagccgggactgtcgggcgtacacaaatcgcccgcagaagcgcggccggccgtctggaccgatggctgtgtagaagtactcgccgatagtggaaaccgacgccccagcactcgtccgggatcctctagcgaccggcatgcccgctgaaatcaccagtctctctctacaaatctatctctctctataataatgtgtgagtagttcccagataagggaattagggttcttatagggtttcgctcatgtgttgagcatataagaaacccttagtatgtatttgtatttgtaaaatacttctatcaataaaatttctaattcctaaaaccaaaatccaggggacgtc

SEQ ID NO: 25 - DNA, 769 bp, Oryza sativa
ccagtgaaagcagtgaattgaagcattcccgaaacccactggaatgatctagtactcactctacgatgtacagtgaagtaatacttcaaaactggtgtaatttggtatgccaaaaggactccatagtttcacgacatatttccaaacggttcaggatcagtactgcccatctgcctggggcccacactagcgggcaattggttctcgtagtttctcgttctcaatcaatcattccatactcgctatcccctccatcacagaataaatgcaacaatgagtttccgtgtacaaatttaatcgttcgtcttatttaaaatattttttaaaaaactaaaaaacaaaagtcacgcataaagtactattcatgttttataatctaataacagtataaatactaatcataaaaaaaaattcaaataagatggacgattaaagttgaacactgaaattcatggctgcttttgttttgagactgagggagtacacgataagatttgatcgcaatcaaagtaacctacatcaaagaagcaagatatgtgggggaaaaatgaatactctagagcaaattaaggtgagccccgctttgtagaggctgatggagtactggagcgacggaagcgaagcagatcgagtgtgctgtaaagcgaaacgagcaagaaccagagaagtccagagatttcaggacagattagttgtgaacctataaatatcctgcctcattccccaacctccatccatcgagccaagactgaagcatttgatcgagctc

SEQ ID NO: 26 - DNA, 3316 bp, Artificial Sequence
  neomycin phosphotransferaseII (nptII) expression unit
gtcattcatatgcttgagaagagagtcgggatagtccaaaataaaacaaaggtaagattacctggtcaaaagtgaaaacatcagttaaaaggtggtataaagtaaaatatcggtaataaaaggtggcccaaagtgaaatttactcttttctactattataaaaattgaggatgtttttgtcggtactttgatacgtcatttttgtatgaattggtttttaagtttattcgcttttggaaatgcatatctgtatttgagtcgggttttaagttcgtttgcttttgtaaatacagagggatttgtataagaaatatctttaaaaaaacccatatgctaatttgacataatttttgagaaaaatatatattcaggcgaattctcacaatgaacaataataagattaaaatagctttcccccgttgcagcgcatgggtattttttctagtaaaaataaaagataaacttagactcaaaacatttacaaaaacaacccctaaagttcctaaagcccaaagtgctatccacgatccatagcaagcccagcccaacccaacccaacccaacccaccccagtccagccaactggacaatagtctccacacccccccactatcaccgtgagttgtccgcacgcaccgcacgtctcgcagccaaaaaaaaaaaaagaaagaaaaaaaagaaaaagaaaaaacagcaggtgggtccgggtcgtgggggccggaaacgcgaggaggatcgcgagccagcgacgaggccggccctccctccgcttccaaagaaacgccccccatcgccactatatacatacccccccctctcctcccatccccccaaccctaccaccaccaccaccaccacctccacctcctcccccctcgctgccggacgacgagctcctcccccctccccctccgccgccgccgcgccggtaaccaccccgcccctctcctctttctttctccgttttttttttccgtctcggtctcgatctttggccttggtagtttgggtgggcgagaggcggcttcgtgcgcgcccagatcggtgcgcgggaggggcgggatctcgcggctggggctctcgccggcgtggatccggcccggatctcgcggggaatggggctctcggatgtagatctgcgatccgccgttgttgggggagatgatggggggtttaaaatttccgccatgctaaacaagatcaggaagaggggaaaagggcactatggtttatatttttatatatttctgctgcttcgtcaggcttagatgtgctagatctttctttcttctttttgtgggtagaatttgaatccctcagcattgttcatcggtagtttttcttttcatgatttgtgacaaatgcagcctcgtgcggagcttttttgtaggtagaccggggggcaatgagatatgattgaacaagatggattgcacgcaggttctccggccgcttgggtggagaggctattcggctatgactgggcacaacagacaatcggctgctctgatgccgccgtgttccggctgtcagcgcaggggcgcccggttctttttgtcaagaccgacctgtccggtgccctgaatgaactgcaggacgaggcagcgcggctatcgtggctggccacgacgggcgttccttgcgcagctgtgctcgacgttgtcactgaagcgggaagggactggctgctattgggcgaagtgccggggcaggatctcctgtcatctcaccttgctcctgccgagaaagtatccatcatggctgatgcaatgcggcggctgcatacgcttgatccggctacctgcccattcgaccaccaagcgaaacatcgcatcgagcgagcacgtactcggatggaagccggtcttgtcgatcaggatgatctggacgaagagcatcaggggctcgcgccagccgaactgttcgccaggctcaaggcgcgcatgcccgacggcgatgatctcgtcgtgacccatggcgatgcctgcttgccgaatatcatggtggaaaatggccgcttttctggattcatcgactgtggccggctgggtgtggcggaccgctatcaggacatagcgttggctacccgtgatattgctgaagagcttggcggcgaatgggctgaccgcttcctcgtgctttacggtatcgccgctcccgattcgcagcgcatcgccttctatcgccttcttgacgagttcttctgagagctctctagatgggctaatctaaaacgatttatctgtggcttcaagtgtatcgatcacttatgtgaggtgtaattactggtgtttttggtgtgctctggttcctttcaagtgtgttgttgccgctcgaactactccgctatgtaaaacggtaaaacctgttgtctcattatgaaagtgaactatattatgttctactactactctacttagtcaattttcttcaccttgattagtgtaaatatgaatcttatattcttatgtcttaagaaattagcacatgtgaagcctccaagtgcatattttctcgatcgcgagacgcacaatgcgtgagaaattcagctggttatactcaaatatattaatatatctagcagcagctcatggagattcaggaaacttggcatccctaatccctaccatttccattcttccgagattgacagttcaatacaagtacagtaatctcctggtaagtttcttattaacttgacatgtagtagtaataatttgtacgtagcatagatacatagacacaaaaatgtcctccccattgagctagccgattggagccgaacaccgcaggaatgaatttacataatctgcaaagaataaatggaatgtgcctccacaggaaaaccagcggcagtgtggcgttttcaagagcagccgtaagtcgaagcctattctgaatcgtagaaatcactggggcatggtgtaattacatccgactccaacatctgtaccaccctgtgcattgtaggccgctcctctggcaaagaacttacacattgtttagcaagagaaagtagagcatccaaggtctcaatctgcactccctcacaatatggatcgacaatttccctctcccgattctcaccgaccaggaaattcaactgccacagagcaagtagattatttcaagaatacattaaatcaattgaaggcatacgtaattcatatcagaaaactgtggatatgaaatggaatgacataaaggtcatacatacccatccaacaatgttcaatcccttttcaataaatgatgcatcagtaggtcgttttccgcttagtatttcaagtagcaaaactccaaaactgtagacgtc

SEQ ID NO: 27 - DNA, 1584 bp, Artificial Sequence
  Enhanced Green Fluorescent Protein (EGFP)  expression unit
ccatggagtcaaagattcaaatagaggacctaacagaactcgccgtaaagactggcgaacagttcatacagagtctcttacgactcaatgacaagaagaaaatcttcgtcaacatggtggagcacgacacacttgtctactccaaaaatatcaaagatacagtctcagaagaccaaagggcaattgagacttttcaacaaagggtaatatccggaaacctcctcggattccattgcccagctatctgtcactttattgtgaagatagtggaaaaggaaggtggctcctacaaatgccatcattgcgataaaggaaaggccatcgttgaagatgcctctgccgacagtggtcccaaagatggacccccacccacgaggagcatcgtggaaaaagaagacgttccaaccacgtcttcaaagcaagtggattgatgtgatatctccactgacgtaagggatgacgcacaatcccactatccttcgcaagacccttcctctatataaggaagttcatttcatttggagaggacagggtacctagggatctatggtgagcaagggcgaggagctgttcaccggggtggtgcccatcctggtcgagctggacggcgacgtaaacggccacaagttcagcgtgtccggcgagggcgagggcgatgccacctacggcaagctgaccctgaagttcatctgcaccaccggcaagctgcccgtgccctggcccaccctcgtgaccaccctgacctacggcgtgcagtgcttcagccgctaccccgaccacatgaagcagcacgacttcttcaagtccgccatgcccgaaggctacgtccaggagcgcaccatcttcttcaaggacgacggcaactacaagacccgcgccgaggtgaagttcgagggcgacaccctggtgaaccgcatcgagctgaagggcatcgacttcaaggaggacggcaacatcctggggcacaagctggagtacaactacaacagccacaacgtctatatcatggccgacaagcagaagaacggcatcaaggtgaacttcaagatccgccacaacatcgaggacggcagcgtgcagctcgccgaccactaccagcagaacacccccatcggcgacggccccgtgctgctgcccgacaaccactacctgagcacccagtccgccctgagcaaagaccccaacgagaagcgcgatcacatggtcctgctggagttcgtgaccgccgccgggatcactctcggcatggacgagctgtacaagtaatctagagttaacctagcttgttcgagtattatggcattgggaaaactgtttttcttgtaccatttgttgtgcttgtaatttactgtgttttttattcggttttcgctatcgaactgtgaaatggaaatggatggagaagagttaatgaatgatatggtccttttgttcattctcaaattaatattatttgttttttctcttatttgttgtgtgttgaatttgaaattataagagatatgcaaacattttgttttgagtaaaaatgtgtcaaatcgtggcctctaatgaccgaagttaatatgaggagtaaaacactag

SEQ ID NO: 28 - DNA, 2659 bp, Artificial Sequence
  hygromycin phosphotransferase (hpt) expression unit
gtcattcatatgcttgagaagagagtcgggatagtccaaaataaaacaaaggtaagattacctggtcaaaagtgaaaacatcagttaaaaggtggtataaagtaaaatatcggtaataaaaggtggcccaaagtgaaatttactcttttctactattataaaaattgaggatgtttttgtcggtactttgatacgtcatttttgtatgaattggtttttaagtttattcgcttttggaaatgcatatctgtatttgagtcgggttttaagttcgtttgcttttgtaaatacagagggatttgtataagaaatatctttaaaaaaacccatatgctaatttgacataatttttgagaaaaatatatattcaggcgaattctcacaatgaacaataataagattaaaatagctttcccccgttgcagcgcatgggtattttttctagtaaaaataaaagataaacttagactcaaaacatttacaaaaacaacccctaaagttcctaaagcccaaagtgctatccacgatccatagcaagcccagcccaacccaacccaacccaacccaccccagtccagccaactggacaatagtctccacacccccccactatcaccgtgagttgtccgcacgcaccgcacgtctcgcagccaaaaaaaaaaaaagaaagaaaaaaaagaaaaagaaaaaacagcaggtgggtccgggtcgtgggggccggaaacgcgaggaggatcgcgagccagcgacgaggccggccctccctccgcttccaaagaaacgccccccatcgccactatatacatacccccccctctcctcccatccccccaaccctaccaccaccaccaccaccacctccacctcctcccccctcgctgccggacgacgagctcctcccccctccccctccgccgccgccgcgccggtaaccaccccgcccctctcctctttctttctccgttttttttttccgtctcggtctcgatctttggccttggtagtttgggtgggcgagaggcggcttcgtgcgcgcccagatcggtgcgcgggaggggcgggatctcgcggctggggctctcgccggcgtggatccggcccggatctcgcggggaatggggctctcggatgtagatctgcgatccgccgttgttgggggagatgatggggggtttaaaatttccgccatgctaaacaagatcaggaagaggggaaaagggcactatggtttatatttttatatatttctgctgcttcgtcaggcttagatgtgctagatctttctttcttctttttgtgggtagaatttgaatccctcagcattgttcatcggtagtttttcttttcatgatttgtgacaaatgcagcctcgtgcggagcttttttgtaggtagaccggggggcaatgagatatgaaaaagcctgaactcaccgcgacgtctgtcgagaagtttctgatcgaaaagttcgacagcgtctccgacctgatgcagctctcggagggcgaagaatctcgtgctttcagcttcgatgtaggagggcgtggatatgtcctgcgggtaaatagctgcgccgatggtttctacaaagatcgttatgtttatcggcactttgcatcggccgcgctcccgattccggaagtgcttgacattggggaattcagcgagagcctgacctattgcatctcccgccgtgcacagggtgtcacgttgcaagacctgcctgaaaccgaactgcccgctgttctgcagccggtcgcggaggccatggatgcgatcgctgcggccgatcttagccagacgagcgggttcggcccattcggaccgcaaggaatcggtcaatacactacatggcgtgatttcatatgcgcgattgctgatccccatgtgtatcactggcaaactgtgatggacgacaccgtcagtgcgtccgtcgcgcaggctctcgatgagctgatgctttgggccgaggactgccccgaagtccggcacctcgtgcacgcggatttcggctccaacaatgtcctgacggacaatggccgcataacagcggtcattgactggagcgaggcgatgttcggggattcccaatacgaggtcgccaacatcttcttctggaggccgtggttggcttgtatggagcagcagacgcgctacttcgagcggaggcatccggagcttgcaggatcgccgcggctccgggcgtatatgctccgcattggtcttgaccaactctatcagagcttggttgacggcaatttcgatgatgcagcttgggcgcagggtcgatgcgacgcaatcgtccgatccggagccgggactgtcgggcgtacacaaatcgcccgcagaagcgcggccggccgtctggaccgatggctgtgtagaagtactcgccgatagtggaaaccgacgccccagcactcgtccgggatcctctagagtcgacctgcaggcatgcccgctgaaatcaccagtctctctctacaaatctatctctctctataataatgtgtgagtagttcccagataagggaattagggttcttatagggtttcgctcatgtgttgagcatataagaaacccttagtatgtatttgtatttgtaaaatacttctatcaataaaatttctaattcctaaaaccaaaatccaggggtacc

SEQ ID NO: 29 - DNA, 750 bp, Artificial Sequence
  mutated  Green Fluorescent Protein (mGFP) gene
tctagaggatccggcccagttggaatgtaggtggtgagcaagggcgaggagctgttcaccggggtggtgcccatcctggtcgagctggacggcgacgtaaacggccacaagttcagcgtgtccggcgagggcgagggcgatgccacctacggcaagctgaccctgaagttcatctgcaccaccggcaagctgcccgtgccctggcccaccctcgtgaccaccttcacctacggcgtgcagtgcttcagccgctaccccgaccacatgaagcagcacgacttcttcaagtccgccatgcccgaaggctacgtccaggagcgcaccatcttcttcaaggacgacggcaactacaagacccgcgccgaggtgaagttcgagggcgacaccctggtgaaccgcatcgagctgaagggcatcgacttcaaggaggacggcaacatcctggggcacaagctggagtacaactacaacagccacaacgtctatatcatggccgacaagcagaagaacggcatcaaggtgaacttcaagatccgccacaacatcgaggacggcagcgtgcagctcgccgaccactaccagcagaacacccccatcggcgacggccccgtgctgctgcccgacaaccactacctgagcacccagtccgccctgagcaaagaccccaacgagaagcgcgatcacatggtcctgctggagttcgtgaccgccgccgggatcactcacggcatggacgagctgtacaagtaa